European Patent Application EP 4 692 337 A1, published February 11, 2026. Title: CAS PROTEIN AND MUTANT THEREOF, AND CORRESPONDING GENE EDITING SYSTEM AND USE THEREOF. Applicant: YOLTECH THERAPEUTICS CO.,LTD. Application EP 24777751.9, filed March 14, 2024. The sequence listing filed with the application follows.

SEQUENCE LISTING (64 sequences)

SEQ ID NO: 1 - protein, 1086 aa, synthetic construct
MIKNQIIGYEVKLDLNDRKRAFVRDTLRYFAQTSDVFRKGLMCLFAGVDPEMISGYLPEGESGDLWCAVNWFRLVDLSEGLVSEERVVDGSELCRRFQDYAGHAPDRQAEIYLTRRSEGDVQYVWADCRAGYRSFCREVGLSPDQMGFDVLALVARGYIKFDKGENDAWGFVSAVFGDGVKEDTKNKIRMLEGMRRAAHAKPATYEELQESALRETGCSDIKQMIREYKSGQQDDKEGVRKSSGGSHAFFVKYFLRGADRVCGPIGEKELELFVSSCDKTLKQKTSCDEAPITHSAVWKRWFKRRIPHTVGSIQEPYSVACDQAMADISSKNCLNARMVSCPDSGSVAERRKKGTKAKKVGSSGVLEMQDKVSSLSSKGVDLAKSVFDSFNDALDRDRKEDEDSCRFEVLRHHLGKLSDLYEIWVKNDCDSGIGLYLEEYEGSIKKQPKEELLRAIYPHRESIKAKEFMDAAHRNDLIQKIESRKAHPTVRGNRGVGYGKSKMRGKIMPQSNMHNGRKAGLNPEMWLEADLLNGERWEKHHLKFHSSQFFDQVYCHKDGLPYTKIPGLPRLARHGMPIGLSISPDDVPLVNRVSGNGRRCPRANKRNLRAVANITHNVELHPETAFEIRSNGEYASISHRVQDVAKKSIEAGDRSLGYDRNQTAQDTYAVLCVVNEGGYAHRGNLVELVAVGKISSKSMKRRTDGSMYECDDLAYDGLPYAEFSEWREERKAFMHRLIPLLPPATKKLGSSREPMDLPKELEALTHCKSLYVWNRRFLIIFRVALKRALKEQASNLFRQEILDICHANLSPLRRSSLSKSGVESLQKLKSLVNAYLSKMKAKREDPLLEADPEFAELFKVITERLKAKRLEKAKRTASDIVRLANLHGCSFVSGESDLPTTSKVNKKFQNASNTDWMARKVEDLVKSMCIRSGIAFRGIDPSYTSLRDPLQFETDGRSVIRCRFWKAENGSAPEYVIDGLVRYTKHAVKNMEQSRPLSSFHRGGLAFCRKYGIDPARLTPKVVRGVLARHEVVYLPRAGGRYFLATLPLVAGAPVFEWDGQQMYVLDADEVAAINIALEAIPSKLP

SEQ ID NO: 2 - DNA, 3258 bp, synthetic construct
  source 1..3258: mol_type = other DNA
atgatcaagaaccaaatcatcggatatgaagtgaagcttgacctcaacgacaggaagagggcttttgttagggataccttgcggtacttcgcccagacatcggatgtgttccgaaagggcctgatgtgcctgttcgctggcgtcgaccccgagatgataagcggctacctgcccgagggggaatccggcgacctgtggtgcgccgtcaactggttccgcctcgtggatctgtcggagggtcttgtctccgaggagcgggtggtagacgggtcggagctgtgccgcaggttccaagactacgcaggtcatgcgcccgaccggcaggcggagatatacctgactaggaggagcgagggcgatgtccagtacgtttgggccgactgccgtgctggctaccgcagcttctgccgtgaggtgggactgagcccagaccagatgggatttgacgtgcttgcgcttgtggcaaggggctacatcaagttcgacaagggcgaaaacgatgcctgggggtttgtatccgccgtcttcggcgacggcgtcaaggaggacaccaagaacaagattcgcatgctcgagggcatgaggagagccgcacacgccaagccggccacctacgaggagcttcaggaatcggcgctgagggagacgggatgcagcgacatcaagcaaatgatcagggagtacaagtccggtcagcaggacgacaaggaaggcgtcagaaaaagcagcggcggcagtcacgcattcttcgtgaaatacttcttgaggggagccgatcgggtatgcggccccatcggcgagaaggagctggaattgttcgtcagtagctgcgacaagaccctgaagcaaaaaacatcgtgcgacgaggcgccgatcacgcacagcgccgtgtggaagaggtggttcaagaggaggataccgcacaccgttggttcaatccaggaaccatacagcgttgcgtgcgaccaagccatggccgacataagctctaagaactgcctgaacgcccgcatggtgagctgcccagacagcggctcggtggccgagcgcaggaagaagggcaccaaggcgaagaaggtcgggtcatccggcgtgctcgagatgcaggacaaggtttcgtccctgtcgagcaagggcgttgatcttgcgaagtccgtattcgacagcttcaacgatgctctggacagggaccgcaaggaggacgaggattcctgccggttcgaggtcctcaggcatcacctcggcaagctttccgacctttacgagatttgggtgaagaacgactgcgactccggcataggtctatatctggaggaatacgaaggttcgattaaaaaacagccgaaagaggaactgctgcgtgcgatctacccgcatcgagagtcaataaaggccaaggagttcatggacgcagcgcaccgcaacgacctcatccaaaagatcgagtcccgcaaggcgcacccgactgtgcgtggcaacaggggcgtcggttacggcaaatccaagatgaggggcaagataatgccgcagtccaacatgcacaacggtcgcaaggccggcctgaaccccgagatgtggctcgaggcggatctcctgaacggggagaggtgggagaaacatcacctgaagttccactcgtcgcagttcttcgatcaggtctactgccacaaggacggactgccctacacgaaaatccctggcctgccgaggttggcacggcacggcatgcccatcgggctgtcgataagccccgatgacgttcctctggtgaaccgtgtgtccggcaacggcaggcgttgcccgagggcgaacaagagaaacctgagggccgtcgccaacatcactcacaacgtggaactccacccggaaacagccttcgagatacgcagcaacggcgaatacgcaagcatcagccacagggtgcaagatgtcgccaagaagagcatcgaggccggcgatcgaagtcttggctacgaccgaaatcagaccgcacaggacacctacgcagtactgtgtgtcgtcaacgagggaggttatgcccacaggggcaacttggtcgagctcgtcgccgtcggcaagatctcgagcaagagcatgaagcgcaggacggacggctcgatgtacgagtgcgacgacctggcctatgacggcttgccttatgcggagttctccgagtggagggaggaacggaaagcattcatgcatcgcctgatcccgctgctgcctccggcaaccaagaagcttggcagcagcagggagccaatggatctgccgaaggaactcgaggccctgacgcactgcaagtcgctgtacgtgtggaaccgcaggttcctgatcatcttccgggtcgcactgaagagggccttgaaggaacaggcgtccaatctgttccgccaggagatactcgacatctgtcacgccaatcttagcccgctgagacgaagcagcttgagcaagtccggagttgaatctcttcagaagctgaagagcctcgtcaacgcctacctcagcaaaatgaaggcgaagagggaggacccactgcttgaggccgacccagagttcgccgagctgttcaaggtaatcaccgagcgtctcaaggcgaaaaggctcgagaaggccaaacgcacagccagcgatatcgtccggctggccaacctgcacggctgctccttcgtctccggcgagtccgacctgccgacgaccagcaaggtcaacaagaaattccagaacgcaagcaacacggactggatggctcgcaaggtcgaggacctcgtcaagagcatgtgcattaggtctggcatcgcctttagaggcatcgacccgtcctacacgagcctgcgtgatccgttacagttcgaaaccgacggcaggagcgtcatccgatgccgtttctggaaggcggaaaatggctcggctccggaatatgtcatcgatggtctggtgcgttacacgaagcacgccgtcaagaacatggagcagtcaaggcccctgtcgtccttccacagaggcgggctggccttctgccgcaagtacggcatcgacccagcgagactgacgcccaaggtcgtccgtggcgtgctggcgaggcacgaggtggtatacttgccacgtgccggcggcaggtacttcctcgccacgctgccgctggtggcgggggctcccgtcttcgagtgggatggccagcagatgtatgtcctcgacgccgacgaggtcgctgcgatcaacatcgcactcgaagccataccttccaagctaccg

SEQ ID NO: 3 - DNA, 8242 bp, synthetic construct
  source 1..8242: mol_type = other DNA
tgagctgataccgctcgccgcagccgaacgaccgagcgcagcgagtcagtgagcgaggaagcggaagagcgcccaatacgcaaaccgcctctccccgcgcgttggccgattcattaatgcagctggcacgacaggtttcccgactggaaagcgggcagtgagcgcaacgcaattaatgtgagttagctcactcattaggcaccccaggctttacactttatgcttccggctcgtatgttgtgtggaattgtgagcggataacaatttcacacaggaaacagctatgaccatgattacgccaagcgcgcaattaaccctcactaaagggaacaaaagctggagctgcaagcttaatgtagtcttatgcaatactcttgtagtcttgcaacatggtaacgatgagttagcaacatgccttacaaggagagaaaaagcaccgtgcatgccgattggtggaagtaaggtggtacgatcgtgccttattaggaaggcaacagacgggtctgacatggattggacgaaccactgaattgccgcattgcagagatattgtatttaagtgcctagctcgatacataaacgggtctctctggttagaccagatctgagcctgggagctctctggctaactagggaacccactgcttaagcctcaataaagcttgccttgagtgcttcaagtagtgtgtgcccgtctgttgtgtgactctggtaactagagatccctcagacccttttagtcagtgtggaaaatctctagcagtggcgcccgaacagggacttgaaagcgaaagggaaaccagaggagctctctcgacgcaggactcggcttgctgaagcgcgcacggcaagaggcgaggggcggcgactggtgagtacgccaaaaattttgactagcggaggctagaaggagagagatgggtgcgagagcgtcagtattaagcgggggagaattagatcgcgatgggaaaaaattcggttaaggccagggggaaagaaaaaatataaattaaaacatatagtatgggcaagcagggagctagaacgattcgcagttaatcctggcctgttagaaacatcagaaggctgtagacaaatactgggacagctacaaccatcccttcagacaggatcagaagaacttagatcattatataatacagtagcaaccctctattgtgtgcatcaaaggatagagataaaagacaccaaggaagctttagacaagatagaggaagagcaaaacaaaagtaagaccaccgcacagcaagcggccgctgatcttcagacctggaggaggagatatgagggacaattggagaagtgaattatataaatataaagtagtaaaaattgaaccattaggagtagcacccaccaaggcaaagagaagagtggtgcagagagaaaaaagagcagtgggaataggagctttgttccttgggttcttgggagcagcaggaagcactatgggcgcagcgtcaatgacgctgacggtacaggccagacaattattgtctggtatagtgcagcagcagaacaatttgctgagggctattgaggcgcaacagcatctgttgcaactcacagtctggggcatcaagcagctccaggcaagaatcctggctgtggaaagatacctaaaggatcaacagctcctggggatttggggttgctctggaaaactcatttgcaccactgctgtgccttggaatgctagttggagtaataaatctctggaacagatttggaatcacacgacctggatggagtgggacagagaaattaacaattacacaagcttaatacactccttaattgaagaatcgcaaaaccagcaagaaaagaatgaacaagaattattggaattagataaatgggcaagtttgtggaattggtttaacataacaaattggctgtggtatataaaattattcataatgatagtaggaggcttggtaggtttaagaatagtttttgctgtactttctatagtgaatagagttaggcagggatattcaccattatcgtttcagacccacctcccaaccccgaggggacccagagagggcctatttcccatgattccttcatatttgcatatacgatacaaggctgttagagagataattagaattaatttgactgtaaacacaaagatattagtacaaaatacgtgacgtagaaagtaataatttcttgggtagtttgcagttttaaaattatgttttaaaatggactatcatatgcttaccgtaacttgaaagtatttcgatttcttggctttatatatcttgtggaaaggacgaaacaccggagacggacgtctctttttttaagcttggcgtaactagatcttgagacaaatggcagtattcatccacaattttaaaagaaaaggggggattggggggtacagtgcaggggaaagaatagtagacataatagcaacagacatacaaactaaagaattacaaaaacaaattacaaaaattcaaaattttcgggtttattacagggacagcagagatccactttggcgccggctcgagggggcccgggtgcaaagatggataaagttttaaacagagaggaatctttgcagctaatggaccttctaggtcttgaaaggagtgggaattggctccggtgcccgtcagtgggcagagcgcacatcgcccacagtccccgagaagttggggggaggggtcggcaattgatccggtgcctagagaaggtggcgcggggtaaactgggaaagtgatgtcgtgtactggctccgcctttttcccgagggtgggggagaaccgtatataagtgcagtagtcgccgtgaacgttctttttcgcaacgggtttgccgccagaacacaggtaagtgccgtgtgtggttcccgcgggcctggcctctttacgggttatggcccttgcgtgccttgaattacttccacctggctgcagtacgtgattcttgatcccgagcttcgggttggaagtgggtgggagagttcgaggccttgcgcttaaggagccccttcgcctcgtgcttgagttgaggcctggcctgggcgctggggccgccgcgtgcgaatctggtggcaccttcgcgcctgtctcgctgctttcgataagtctctagccatttaaaatttttgatgacctgctgcgacgctttttttctggcaagatagtcttgtaaatgcgggccaagatctgcacactggtatttcggtttttggggccgcgggcggcgacggggcccgtgcgtcccagcgcacatgttcggcgaggcggggcctgcgagcgcggccaccgagaatcggacgggggtagtctcaagctggccggcctgctctggtgcctggcctcgcgccgccgtgtatcgccccgccctgggcggcaaggctggcccggtcggcaccagttgcgtgagcggaaagatggccgcttcccggccctgctgcagggagctcaaaatggaggacgcggcgctcgggagagcgggcgggtgagtcacccacacaaaggaaaagggcctttccgtcctcagccgtcgcttcatgtgactccacggagtaccgggcgccgtccaggcacctcgattagttctcgagcttttggagtacgtcgtctttaggttggggggaggggttttatgcgatggagtttccccacactgagtgggtggagactgaagttaggccagcttggcacttgatgtaattctccttggaatttgccctttttgagtttggatcttggttcattctcaagcctcagacagtggttcaaagtttttttcttccatttcaggtgtcgtgacgtacggccaccatgaccgagtacaagcccacggtgcgcctcgccacccgcgacgacgtccccagggccgtacgcaccctcgccgccgcgttcgccgactaccccgccacgcgccacaccgtcgatccggaccgccacatcgagcgggtcaccgagctgcaagaactcttcctcacgcgcgtcgggctcgacatcggcaaggtgtgggtcgcggacgacggcgccgccgtggcggtctggaccacgccggagagcgtcgaagcgggggcggtgttcgccgagatcggcccgcgcatggccgagttgagcggttcccggctggccgcgcagcaacagatggaaggcctcctggcgccgcaccggcccaaggagcccgcgtggttcctggccaccgtcggagtctcgcccgaccaccagggcaagggtctgggcagcgccgtcgtgctccccggagtggaggcggccgagcgcgccggggtgcccgccttcctggagacctccgcgccccgcaacctccccttctacgagcggctcggcttcaccgtcaccgccgacgtcgaggtgcccgaaggaccgcgcacctggtgcatgacccgcaagcccggtgcctgaacgcgttaagtcgacaatcaacctctggattacaaaatttgtgaaagattgactggtattcttaactatgttgctccttttacgctatgtggatacgctgctttaatgcctttgtatcatgctattgcttcccgtatggctttcattttctcctccttgtataaatcctggttgctgtctctttatgaggagttgtggcccgttgtcaggcaacgtggcgtggtgtgcactgtgtttgctgacgcaacccccactggttggggcattgccaccacctgtcagctcctttccgggactttcgctttccccctccctattgccacggcggaactcatcgccgcctgccttgcccgctgctggacaggggctcggctgttgggcactgacaattccgtggtgttgtcggggaaatcatcgtcctttccttggctgctcgcctgtgttgccacctggattctgcgcgggacgtccttctgctacgtcccttcggccctcaatccagcggaccttccttcccgcggcctgctgccggctctgcggcctcttccgcgtcttcgccttcgccctcagacgagtcggatctccctttgggccgcctccccgcgtcgactttaagaccaatgacttacaaggcagctgtagatcttagccactttttaaaagaaaaggggggactggaagggctaattcactcccaacgaagacaagatctgctttttgcttgtactgggtctctctggttagaccagatctgagcctgggagctctctggctaactagggaacccactgcttaagcctcaataaagcttgccttgagtgcttcaagtagtgtgtgcccgtctgttgtgtgactctggtaactagagatccctcagacccttttagtcagtgtggaaaatctctagcagtacgtatagtagttcatgtcatcttattattcagtatttataacttgcaaagaaatgaatatcagagagtgagaggaacttgtttattgcagcttataatggttacaaataaagcaatagcatcacaaatttcacaaataaagcatttttttcactgcattctagttgtggtttgtccaaactcatcaatgtatcttatcatgtctggctctagctatcccgcccctaactccgcccatcccgcccctaactccgcccagttccgcccattctccgccccatggctgactaattttttttatttatgcagaggccgaggccgcctcggcctctgagctattccagaagtagtgaggaggcttttttggaggcctagggacgtacccaattcgccctatagtgagtcgtattacgcgcgctcactggccgtcgttttacaacgtcgtgactgggaaaaccctggcgttacccaacttaatcgccttgcagcacatccccctttcgccagctggcgtaatagcgaagaggcccgcaccgatcgcccttcccaacagttgcgcagcctgaatggcgaatgggacgcgccctgtagcggcgcattaagcgcggcgggtgtggtggttacgcgcagcgtgaccgctacacttgccagcgccctagcgcccgctcctttcgctttcttcccttcctttctcgccacgttcgccggctttccccgtcaagctctaaatcgggggctccctttagggttccgatttagtgctttacggcacctcgaccccaaaaaacttgattagggtgatggttcacgtagtgggccatcgccctgatagacggtttttcgccctttgacgttggagtccacgttctttaatagtggactcttgttccaaactggaacaacactcaaccctatctcggtctattcttttgatttataagggattttgccgatttcggcctattggttaaaaaatgagctgatttaacaaaaatttaacgcgaattttaacaaaatattaacgcttacaatttaggtggcacttttcggggaaatgtgcgcggaacccctatttgtttatttttctaaatacattcaaatatgtatccgctcatgagacaataaccctgataaatgcttcaataatattgaaaaaggaagagtatgagtattcaacatttccgtgtcgcccttattcccttttttgcggcattttgccttcctgtttttgctcacccagaaacgctggtgaaagtaaaagatgctgaagatcagttgggtgcacgagtgggttacatcgaactggatctcaacagcggtaagatccttgagagttttcgccccgaagaacgttttccaatgatgagcacttttaaagttctgctatgtggcgcggtattatcccgtattgacgccgggcaagagcaactcggtcgccgcatacactattctcagaatgacttggttgagtactcaccagtcacagaaaagcatcttacggatggcatgacagtaagagaattatgcagtgctgccataaccatgagtgataacactgcggccaacttacttctgacaacgatcggaggaccgaaggagctaaccgcttttttgcacaacatgggggatcatgtaactcgccttgatcgttgggaaccggagctgaatgaagccataccaaacgacgagcgtgacaccacgatgcctgtagcaatggcaacaacgttgcgcaaactattaactggcgaactacttactctagcttcccggcaacaattaatagactggatggaggcggataaagttgcaggaccacttctgcgctcggcccttccggctggctggtttattgctgataaatctggagccggtgagcgtgggtctcgcggtatcattgcagcactggggccagatggtaagccctcccgtatcgtagttatctacacgacggggagtcaggcaactatggatgaacgaaatagacagatcgctgagataggtgcctcactgattaagcattggtaactgtcagaccaagtttactcatatatactttagattgatttaaaacttcatttttaatttaaaaggatctaggtgaagatcctttttgataatctcatgaccaaaatcccttaacgtgagttttcgttccactgagcgtcagaccccgtagaaaagatcaaaggatcttcttgagatcctttttttctgcgcgtaatctgctgcttgcaaacaaaaaaaccaccgctaccagcggtggtttgtttgccggatcaagagctaccaactctttttccgaaggtaactggcttcagcagagcgcagataccaaatactgttcttctagtgtagccgtagttaggccaccacttcaagaactctgtagcaccgcctacatacctcgctctgctaatcctgttaccagtggctgctgccagtggcgataagtcgtgtcttaccgggttggactcaagacgatagttaccggataaggcgcagcggtcgggctgaacggggggttcgtgcacacagcccagcttggagcgaacgacctacaccgaactgagatacctacagcgtgagctatgagaaagcgccacgcttcccgaagggagaaaggcggacaggtatccggtaagcggcagggtcggaacaggagagcgcacgagggagcttccagggggaaacgcctggtatctttatagtcctgtcgggtttcgccacctctgacttgagcgtcgatttttgtgatgctcgtcaggggggcggagcctatggaaaaacgccagcaacgcggcctttttacggttcctggccttttgctggccttttgctcacatgttctttcctgcgttatcccctgattctgtggataaccgtattaccgcctttgag

SEQ ID NO: 4 - DNA, 6161 bp, synthetic construct
  source 1..6161: mol_type = other DNA
acaccatcgaatggtgcaaaacctttcgcggtatggcatgatagcgcccggaagagagtcaattcagggtggtgaatgtgaaaccagtaacgttatacgatgtcgcagagtatgccggtgtctcttatcagaccgtttcccgcgtggtgaaccaggccagccacgtttctgcgaaaacgcgggaaaaagtggaagcggcgatggcggagctgaattacattcccaaccgcgtggcacaacaactggcgggcaaacagtcgttgctgattggcgttgccacctccagtctggccctgcacgcgccgtcgcaaattgtcgcggcgattaaatctcgcgccgatcaactgggtgccagcgtggtggtgtcgatggtagaacgaagcggcgtcgaagcctgtaaagcggcggtgcacaatcttctcgcgcaacgcgtcagtgggctgatcattaactatccgctggatgaccaggatgccattgctgtggaagctgcctgcactaatgttccggcgttatttcttgatgtctctgaccagacacccatcaacagtattattttctcccatgaagacggtacgcgactgggcgtggagcatctggtcgcattgggtcaccagcaaatcgcgctgttagcgggcccattaagttctgtctcggcgcgtctgcgtctggctggctggcataaatatctcactcgcaatcaaattcagccgatagcggaacgggaaggcgactggagtgccatgtccggttttcaacaaaccatgcaaatgctgaatgagggcatcgttcccactgcgatgctggttgccaacgatcagatggcgctgggcgcaatgcgcgccattaccgagtccgggctgcgcgttggtgcggatatctcggtagtgggatacgacgataccgaagacagctcatgttatatcccgccgttaaccaccatcaaacaggattttcgcctgctggggcaaaccagcgtggaccgcttgctgcaactctctcagggccaggcggtgaagggcaatcagctgttgcccgtctcactggtgaaaagaaaaaccaccctggcgcccaatacgcaaaccgcctctccccgcgcgttggccgattcattaatgcagctggcacgacaggtttcccgactggaaagcgggcagtgagcgcaacgcaattaatgtaagttagctcaaatattctgaaatgagctgttgacaattaatcatcggctcgtataatgtgtggaattgtgagcggataacaatttcacacaggaaacagaattctttgcatctccccattccatgagcatatgcgatcttccccatcggtgatgtcggcgatataggcgccagcaaccgcacctgtggcgccggtgatgccggccacgatgcgtccggcgtagaggatctgctcatgtttgacagcttatcatcgatgcataatgtgcctgtcaaatggacgaagcagggattctgcaaaccctatgctactccgtcaagccgtcaattgtctgattcgttaccaattatgacaacttgacggctacatcattcactttttcttcacaaccggcacggaactcgctcgggctggccccggtgcattttttaaatacccgcgagaaatagagttgatcgtcaaaaccaacattgcgaccgacggtggcgataggcatccgggtggtgctcaaaagcagcttcgcctggctgatacgttggtcctcgcgccagcttaagacgctaatccctaactgctggcggaaaagatgtgacagacgcgacggcgacaagcaaacatgctgtgcgacgctggcgatatcaaaattgctgtctgccaggtgatcgctgatgtactgacaagcctcgcgtacccgattatccatcggtggatggagcgactcgttaatcgcttccatgcgccgcagtaacaattgctcaagcagatttatcgccagcagctccgaatagcgcccttccccttgcccggcgttaatgatttgcccaaacaggtcgctgaaatgcggctggtgcgcttcatccgggcgaaagaaccccgtattggcaaatattgacggccagttaagccattcatgccagtaggcgcgcggacgaaagtaaacccactggtgataccattcgcgagcctccggatgacgaccgtagtgatgaatctctcctggcgggaacagcaaaatatcacccggtcggcaaacaaattctcgtccctgatttttcaccaccccctgaccgcgaatggtgagattgagaatataacctttcattcccagcggtcggtcgataaaaaaatcgagataaccgttggcctcaatcggcgttaaacccgccaccagatgggcattaaacgagtatcccggcagcaggggatcattttgcgcttcagccatacttttcatactcccgccattcagagaagaaaccaattgtccatattgcatcagacattgccgtcactgcgtcttttactggctcttctcgctaaccaaaccggtaaccccgcttattaaaagcattctgtaacaaagcgggaccaaagccatgacaaaaacgcgtaacaaaagtgtctataatcacggcagaaaagtccacattgattatttgcacggcgtcacactttgctatgccatagcatttttatccataagattagcggatcctacctgacgctttttatcgcaactctctactgtttctccatacccgtttttttgggctagcgaattcgagctcatgcagtttaaggtttacacctataaaagagagagccgttatcgtctgtttgtggatgtacagagtgatattattgacacgcccgggcgacggatggtgatccccctggccagtgcacgtctgctgtcagataaagtctcccgtgaactttacccggtggtgcatatcggggatgaaagctggcgcatgatgaccaccgatatggccagtgtgccggtatccgttatcggggaagaagtggctgatctcagccaccgcgaaaatgacatcaaaaacgccattaacctgatgttctggggaatataatctagagtcgacctgcaggcatgcaagcttggctgttttggcggatgagagaagattttcagcctgatacagattaaatcagaacgcagaagcggtctgataaaacagaatttgcctggcggcagtagcgcggtggtcccacctgaccccatgccgaactcagaagtgaaacgccgtagcgccgatggtagtgtggggtctccccatgcgagagtagggaactgccaggcatcaaataaaacgaaaggctcagtcgaaagactgggcctttcgttttatctgttgtttgtcggtgaacgctctcctgagtaggacaaatccgccgggagcggatttgaacgttgcgaagcaacggcccggagggtggcgggcaggacgcccgccataaactgccaggcatcaaattaagcagaaggccatcctgacggatggcctttttgcgtttctacaaactctggatcctccggcgttcagcctgtgccacagccgacaggatggtgaccaccatttgccccatatcaccgtcggtactgatcccgtcgtcaataaaccgaaccgctacaccctgagcatcaaactcttttatcagttggatcatgtcggcggtgtcgcggccaagacggtcgagcttcttcaccagaatgacatcaccttcctccaccttcatcctcagcaaatccagcccttcccgatctgttgaactgccggatgccttgtcggtaaagatgcggttagcttttacccctgcatctttgagcgctgaggtctgcctcgtgaagaaggtgttgctgactcataccaggcctgaatcgccccatcatccagccagaaagtgagggagccacggttgatgagagctttgttgtaggtggaccagttggtgattttgaacttttgctttgccacggaacggtctgcgttgtcgggaagatgcgtgatctgatccttcaactcagcaaaagttcgatttattcaacaaagccgccgtcccgtcaagtcagcgtaatgctctgccagtgttacaaccaattaaccaattctgattagaaaaactcatcgagcatcaaatgaaactgcaatttattcatatcaggattatcaataccatatttttgaaaaagccgtttctgtaatgaaggagaaaactcaccgaggcagttccataggatggcaagatcctggtatcggtctgcgattccgactcgtccaacatcaatacaacctattaatttcccctcgtcaaaaataaggttatcaagtgagaaatcaccatgagtgacgactgaatccggtgagaatggcaaaagcttatgcatttctttccagacttgttcaacaggccagccattacgctcgtcatcaaaatcactcgcatcaaccaaaccgttattcattcgtgattgcgcctgagcgagacgaaatacgcgatcgctgttaaaaggacaattacaaacaggaatcgaatgcaaccggcgcaggaacactgccagcgcatcaacaatattttcacctgaatcaggatattcttctaatacctggaatgctgttttcccggggatcgcagtggtgagtaaccatgcatcatcaggagtacggataaaatgcttgatggtcggaagaggcataaattccgtcagccagtttagtctgaccatctcatctgtaacatcattggcaacgctacctttgccatgtttcagaaacaactctggcgcatcgggcttcccatacaatcgatagattgtcgcacctgattgcccgacattatcgcgagcccatttatacccatataaatcagcatccatgttggaatttaatcgcggcctcgagcaagacgtttcccgttgaatatggctcataacaccccttgtattactgtttatgtaagcagacagttttattgttcatgatgatatatttttatcttgtgcaatgtaacatcagagattttgagacacaacgtggctttgttgaataaatcgaacttttgctgagttgaaggatcagatcacgcatcttcccgacaacgcagaccgttccgtggcaaagcaaaagttcaaaatcaccaactggtccacctacaacaaagctctcatcaaccgtggctccctcactttctggctggatgatggggcgattcaggcctggtatgagtcagcaacaccttcttcacgaggcagacctcagcgctagcggagtgtatactggcttactatgttggcactgatgagggtgtcagtgaagtgcttcatgtggcaggagaaaaaaggctgcaccggtgcgtcagcagaatatgtgatacaggatatattccgcttcctcgctcactgactcgctacgctcggtcgttcgactgcggcgagcggaaatggcttacgaacggggcggagatttcctggaagatgccaggaagatacttaacagggaagtgagagggccgcggcaaagccgtttttccataggctccgcccccctgacaagcatcacgaaatctgacgctcaaatcagtggtggcgaaacccgacaggactataaagataccaggcgtttccccctggcggctccctcgtgcgctctcctgttcctgcctttcggtttaccggtgtcattccgctgttatggccgcgtttgtctcattccacgcctgacactcagttccgggtaggcagttcgctccaagctggactgtatgcacgaaccccccgttcagtccgaccgctgcgccttatccggtaactatcgtcttgagtccaacccggaaagacatgcaaaagcaccactggcagcagccactggtaattgatttagaggagttagtcttgaagtcatgcgccggttaaggctaaactgaaaggacaagttttggtgactgcgctcctccaagccagttacctcggttcaaagagttggtagctcagagaaccttcgaaaaaccgccctgcaaggcggttttttcgttttcagagcaagagattacgcgcagaccaaaacgatctcaagaagatcatcttattaaggggtctgacgctcagtggaacgaaaactcacgttaagggattttggtcatgagattatcaaaaaggatcttcacctagatccttttggtcg

SEQ ID NO: 5 - DNA, 25 bp, synthetic construct
  source 1..25: mol_type = other DNA
tatccatcgtgccgcctcttggcac

SEQ ID NO: 6 - DNA, 20 bp, synthetic construct
  source 1..20: mol_type = other DNA
gcatctccccattccatgag

SEQ ID NO: 7 - DNA, 126 bp, synthetic construct
  source 1..126: mol_type = other DNA
caattgtaatacgactcactataggcaccgtatccatcgtgccgcctcttggcacgcatctccccattccatgagttttttaagcttggcgtagaaggccatcctgacggatggccttttacgcgt

SEQ ID NO: 8 - DNA, 45 bp, synthetic construct
  source 1..45: mol_type = other DNA
tatccatcgtgccgcctcttggcacgcatctccccattccatgag

SEQ ID NO: 9 - DNA, 20 bp, synthetic construct
  source 1..20: mol_type = other DNA
aactgaggaggaatttgtag

SEQ ID NO: 10 - DNA, 20 bp, synthetic construct
  source 1..20: mol_type = other DNA
caaaagcaaaaaccaaaacc

SEQ ID NO: 11 - DNA, 2226 bp, synthetic construct
  source 1..2226: mol_type = other DNA
tttgcatctccccattccatgagcatatgcgatcttccccatcggtgatgtcggcgatataggcgccagcaaccgcacctgtggcgccggtgatgccggccacgatgcgtccggcgtagaggatctgctcatgtttgacagcttatcatcgatgcataatgtgcctgtcaaatggacgaagcagggattctgcaaaccctatgctactccgtcaagccgtcaattgtctgattcgttaccaattatgacaacttgacggctacatcattcactttttcttcacaaccggcacggaactcgctcgggctggccccggtgcattttttaaatacccgcgagaaatagagttgatcgtcaaaaccaacattgcgaccgacggtggcgataggcatccgggtggtgctcaaaagcagcttcgcctggctgatacgttggtcctcgcgccagcttaagacgctaatccctaactgctggcggaaaagatgtgacagacgcgacggcgacaagcaaacatgctgtgcgacgctggcgatatcaaaattgctgtctgccaggtgatcgctgatgtactgacaagcctcgcgtacccgattatccatcggtggatggagcgactcgttaatcgcttccatgcgccgcagtaacaattgctcaagcagatttatcgccagcagctccgaatagcgcccttccccttgcccggcgttaatgatttgcccaaacaggtcgctgaaatgcggctggtgcgcttcatccgggcgaaagaaccccgtattggcaaatattgacggccagttaagccattcatgccagtaggcgcgcggacgaaagtaaacccactggtgataccattcgcgagcctccggatgacgaccgtagtgatgaatctctcctggcgggaacagcaaaatatcacccggtcggcaaacaaattctcgtccctgatttttcaccaccccctgaccgcgaatggtgagattgagaatataacctttcattcccagcggtcggtcgataaaaaaatcgagataaccgttggcctcaatcggcgttaaacccgccaccagatgggcattaaacgagtatcccggcagcaggggatcattttgcgcttcagccatacttttcatactcccgccattcagagaagaaaccaattgtccatattgcatcagacattgccgtcactgcgtcttttactggctcttctcgctaaccaaaccggtaaccccgcttattaaaagcattctgtaacaaagcgggaccaaagccatgacaaaaacgcgtaacaaaagtgtctataatcacggcagaaaagtccacattgattatttgcacggcgtcacactttgctatgccatagcatttttatccataagattagcggatcctacctgacgctttttatcgcaactctctactgtttctccatacccgtttttttgggctagcgaattcgagctcatgcagtttaaggtttacacctataaaagagagagccgttatcgtctgtttgtggatgtacagagtgatattattgacacgcccgggcgacggatggtgatccccctggccagtgcacgtctgctgtcagataaagtctcccgtgaactttacccggtggtgcatatcggggatgaaagctggcgcatgatgaccaccgatatggccagtgtgccggtatccgttatcggggaagaagtggctgatctcagccaccgcgaaaatgacatcaaaaacgccattaacctgatgttctggggaatataatctagagtcgacctgcaggcatgcaagcttggctgttttggcggatgagagaagattttcagcctgatacagattaaatcagaacgcagaagcggtctgataaaacagaatttgcctggcggcagtagcgcggtggtcccacctgaccccatgccgaactcagaagtgaaacgccgtagcgccgatggtagtgtggggtctccccatgcgagagtagggaactgccaggcatcaaataaaacgaaaggctcagtcgaaagactgggcctttcgttttatctgttgtttgtcggtgaacgctctcctgagtaggacaaatccgccgggagcggatttgaacgttgcgaagcaacggcccggagggtggcgggcaggacgcccgccataaactgccaggcatcaaattaagcagaaggccatcctgacggatggcctttttgcgtttctacaaactct

SEQ ID NO: 12 - protein, 1230 aa, synthetic construct
MSKLEKFTNCYSLSKTLRFKAIPVGKTQENIDNKRLLVEDEKRAEDYKGVKKLLDRYYLSFINDVLHSIKLKNLNNYISLFRKKTRTEKENKELENLEINLRKEIAKAFKGNEGYKSLFKKDIIETILPEFLDDKDEIALVNSFNGFTTAFTGFFDNRENMFSEEAKSTSIAFRCINENLTRYISNMDIFEKVDAIFDKHEVQEIKEKILNSDYDVEDFFEGEFFNFVLTQEGIDVYNAIIGGFVTESGEKIKGLNEYINLYNQKTKQKLPKFKPLYKQVLSDRESLSFYGEGYTSDEEVLEVFRNTLNKNSEIFSSIKKLEKLFKNFDEYSSAGIFVKNGPAISTISKDIFGEWNVIRDKWNAEYDDIHLKKKAVVTEKYEDDRRKSFKKIGSFSLEQLQEYADADLSVVEKLKEIIIQKVDEIYKVYGSSEKLFDADFVLEKSLKKNDAVVAIMKDLLDSVKSFENYIKAFFGEGKETNRDESFYGDFVLAYDILLKVDHIYDAIRNYVTQKPYSKDKFKLYFQNPQFMGGWDKDKETDYRATILRYGSKYYLAIMDKKYAKCLQKIDKDDVNGNYEKINYKLLPGPNKMLPKVFFSKKWMAYYNPSEDIQKIYKNGTFKKGDMFNLNDCHKLIDFFKDSISRYPKWSNAYDFNFSETEKYKDIAGFYREVEEQGYKVSFESASKKEVDKLVEEGKLYMFQIYNKDFSDKSHGTPNLHTMYFKLLFDENNHGQIRLSGGAELFMRRASLKKEELVVHPANSPIANKNPDNPKKTTTLSYDVYKDKRFSEDQYELHIPIAINKCPKNIFKINTEVRVLLKHDDNPYVIGIDRGERNLLYIVVVDGKGNIVEQYSLNEIINNFNGIRIKTDYHSLLDKKEKERFEARQNWTSIENIKELKAGYISQVVHKICELVEKYDAVIALEDLNSGFKNSRVKVEKQVYQKFEKMLIDKLNYMVDKKSNPCATGGALKGYQITNKFESFKSMSTQNGFIFYIPAWLTSKIDPSTGFVNLLKTKYTSIADSKKFISSFDRIMYVPEEDLFEFALDYKNFSRTDADYIKKWKLYSYGNRIRIFRNPKKNNVFDWEEVCLTSAYKELFNKYGINYQQGDIRALLCEQSDKAFYSSFMALMSLMLQMRNSITGRTDVDFLISPVKNSDGIFYDSRNYEAQENAILPKNADANGAYNIARKVLWAIGQFKKAEDEKLDKVKIAISNKEWLEYAQTSVKHGS

SEQ ID NO: 13 - DNA, 3690 bp, synthetic construct
  source 1..3690: mol_type = other DNA
atgtcaaagctggagaaattcaccaactgttatagcctgtctaagaccctgcgcttcaaggcaatcccagtgggcaagacacaagagaacattgacaacaaacggctcctggtggaggatgagaagagggctgaagattacaagggcgttaagaagctgctggataggtactatctgtcattcatcaacgatgtcctccacagtatcaagctgaagaatctgaacaattacatttctctgttccggaagaagacacggaccgagaaggagaacaaagagctggagaatctggagatcaacctgaggaaagaaatagctaaggctttcaaagggaacgagggttacaagtccctgttcaagaaagacattatcgagactattctgcctgagttcctggacgataaagatgagatcgccctcgtcaattccttcaatgggtttaccacagcctttaccggcttcttcgacaatagagagaatatgttctctgaagaggccaaatccactagcatcgcctttcgctgcataaacgagaacctgactaggtacatcagcaatatggacatctttgagaaagtcgatgccatattcgacaaacatgaggtgcaggagattaaggagaagatcctgaactcagattacgatgtcgaagatttcttcgagggagagttcttcaacttcgtgctcacacaagagggcattgatgtgtacaatgcaatcattggagggttcgtgacagagagtggcgagaagataaagggcctgaacgagtatatcaacctctacaaccagaaaaccaagcagaaactgcctaagttcaagccactgtacaaacaagtgctctcagatagggaaagcctgagcttctacggtgaagggtatacatcagatgaagaagtgctcgaagtgttccgcaacaccctcaataagaacagtgaaatcttctcttcaatcaagaagctggagaaactgttcaagaatttcgatgagtactcctctgccggaatctttgtgaagaatggccctgcaatatccactattagcaaagacatctttggcgagtggaacgttatcagggataagtggaatgccgagtacgatgatattcatctcaagaagaaagccgtggttacagagaaatacgaggatgatagacgcaagagctttaagaagattggtagcttctctctcgaacagctgcaggagtacgccgacgctgacctgtcagtcgtggagaaactcaaggagatcataatccagaaggtggatgaaatctacaaagtgtatggaagctctgagaaactcttcgatgcagactttgttctggagaagagtctgaagaagaacgacgcagtggttgctatcatgaaggacctgctggattctgttaagtctttcgagaattacattaaggcattctttggtgaagggaaggagacaaatagggacgagagcttctatggcgactttgttctggcctacgacatcctcctcaaggttgaccacatctatgacgctatacggaattacgttacccagaagccctatagcaaagacaagttcaagctgtatttccagaatccacagtttatgggtgggtgggataaagacaaagaaacagattacagggccactatcctgcggtacggcagcaaatactatctggctatcatggataagaagtacgccaaatgcctccagaagatcgacaaggacgacgtgaacggtaactacgagaagatcaattacaagctcctgccaggacctaacaagatgctgcccaaggtgttcttctccaagaaatggatggcctactataacccaagcgaggacattcagaagatatacaagaatgggacattcaagaagggcgatatgttcaacctcaacgactgccacaagctgattgatttcttcaaggatagcatttctcgctatcccaagtggtctaatgcatacgatttcaacttcagcgagactgagaagtacaaagacatcgctggcttctaccgggaggtggaagagcaaggctataaggtgtcattcgaatccgcttctaagaaggaagtggataagctcgtggaagagggtaagctgtacatgttccagatatacaacaaagacttcagcgataagagccacggcactccaaacctccatactatgtatttcaagctgctgtttgacgagaacaaccacggacagattaggctgtcaggaggcgcagaactcttcatgcgcagagcttcactgaagaaggaggaactcgttgtccacccagccaatagccctatagccaataagaatccagacaatcctaagaaaaccactactctgtcttacgatgtgtataaggataagagattctctgaagatcagtacgaactgcacatacccattgccattaacaagtgccctaagaacatcttcaagattaacacagaggttagagtgctcctgaaacacgacgataacccttatgttataggcattgatcgcggagagagaaacctgctgtacatcgtcgtggtggacggcaaaggcaacatcgtggaacagtacagtctcaatgaaatcattaacaatttcaacggaatccgcattaagaccgactaccattctctcctcgacaagaaggagaaagaaaggttcgaagcaagacagaattggacaagtatagagaatatcaaagaactgaaggctgggtacatctctcaggttgtgcacaagatatgtgagctggtggagaagtacgacgctgttatcgccctcgaggacctgaatagcggcttcaagaactccagggtgaaggtggagaagcaggtgtatcagaagttcgagaagatgctgatcgacaagctcaactatatggtggacaagaaatccaatccttgcgctactggtggagccctgaagggctatcaaatcaccaataagttcgaatctttcaagtctatgagcacccagaatggcttcatcttctacatacccgcatggctgacatccaagattgatccctctaccggatttgttaatctgctcaagactaagtacacctctattgctgactcaaagaagttcatatcatcatttgaccgcatcatgtacgtgccagaagaggacctgttcgagtttgccctggattacaagaatttctctcggactgacgccgactacatcaagaagtggaagctctactcttatggtaatcggattcgcatattccgcaatcccaagaagaataacgtgttcgattgggaggaagtttgcctcaccagcgcttacaaggagctgttcaataagtatgggattaactaccagcagggcgacataagagccctgctgtgcgaacaatctgataaggcattctattcctctttcatggcactgatgtcactgatgctgcaaatgcgcaattccatcaccggaagaacagacgtggactttctgatctctcctgtcaagaactcagatggcatcttctacgattcccgcaactatgaagcacaggagaatgctatcctgcctaagaatgccgatgcaaatggagcctataacatcgccagaaaggtcctctgggccataggacaattcaagaaagctgaagatgagaagctggacaaggtgaagatcgccatttcaaacaaagagtggctcgaatatgctcagacctcagtgaagcatggatca

SEQ ID NO: 14 - DNA, 122 bp, synthetic construct
  source 1..122: mol_type = other DNA
caattgtaatacgactcactataggcaccgtaatttctactaagtgtagatgcatctccccattccatgagttttttaagcttggcgtagaaggccatcctgacggatggccttttacgcgt

SEQ ID NO: 15 - DNA, 41 bp, synthetic construct
  source 1..41: mol_type = other DNA
taatttctactaagtgtagatgcatctccccattccatgag

SEQ ID NO: 16 - DNA, 49 bp, synthetic construct
  source 1..49: mol_type = other DNA
cacctatccatcgtgccgcctcttggcacgcatctccccattccatgag

SEQ ID NO: 17 - DNA, 49 bp, synthetic construct
  source 1..49: mol_type = other DNA
aaaactcatggaatggggagatgcgtgccaagaggcggcacgatggata

SEQ ID NO: 18 - DNA, 45 bp, synthetic construct
  source 1..45: mol_type = other DNA
cacctaatttctactaagtgtagatgcatctccccattccatgag

SEQ ID NO: 19 - DNA, 45 bp, synthetic construct
  source 1..45: mol_type = other DNA
aaaactcatggaatggggagatgcatctacacttagtagaaatta

SEQ ID NO: 20 - DNA, 45 bp, synthetic construct
  source 1..45: mol_type = other DNA
tatccatcgtgccgcctcttggcactatatcccttctacaaattc

SEQ ID NO: 21 - DNA, 45 bp, synthetic construct
  source 1..45: mol_type = other DNA
tatccatcgtgccgcctcttggcacgtgtctatttccactttgta

SEQ ID NO: 22 - DNA, 49 bp, synthetic construct
  source 1..49: mol_type = other DNA
cacctatccatcgtgccgcctcttggcactatatcccttctacaaattc

SEQ ID NO: 23 - DNA, 49 bp, synthetic construct
  source 1..49: mol_type = other DNA
aaaagaatttgtagaagggatatagtgccaagaggcggcacgatggata

SEQ ID NO: 24 - DNA, 49 bp, synthetic construct
  source 1..49: mol_type = other DNA
cacctatccatcgtgccgcctcttggcacgtgtctatttccactttgta

SEQ ID NO: 25 - DNA, 49 bp, synthetic construct
  source 1..49: mol_type = other DNA
aaaatacaaagtggaaatagacacgtgccaagaggcggcacgatggata

SEQ ID NO: 26 - DNA, 20 bp, synthetic construct
  source 1..20: mol_type = other DNA
gggtgtattactttgccatg

SEQ ID NO: 27 - DNA, 24 bp, synthetic construct
  source 1..24: mol_type = other DNA
aacctttggtcattcatcaccttc

SEQ ID NO: 28 - protein, 170 aa, synthetic construct
MSELNDAYWMKQALALAQKAREQGEVPVGAILVLDDEVIGQGWNRAITLHDPTAHAEIMALQQGGQIVQNYRLLNATLYVTFEPCVMCAGAMVHSRIKRLVYGVSNSKRGAAGSLLNVLNYPGMNHQIEITAGVMANECSEMLCQFYQQPREVFNAEREARRLNQPDRAD

SEQ ID NO: 29 - protein, 170 aa, synthetic construct
MSELNDAYWMKQALALAQKAREQGEVPVGAILVLDDEVIGQGWNRAITLHDPTAHAEIMALQQGGQIVQNYRLLNATLYVTFEPCVMCAGAMVHSRIKRLVYGVSNSKRGAAGSLLNVLNYPGMNHQIEITAGVMANECSEMLCQFYGMRREVFNAEREARRLNQPDRAD

SEQ ID NO: 30 - DNA, 510 bp, synthetic construct
  source 1..510: mol_type = other DNA
atgagtgagctgaatgatgcttactggatgaaacaggcactcgctttagctcagaaggcccgggaacagggagaagttccagtgggcgctattctggtgctggatgatgaagtgataggacagggatggaatagagccatcaccctgcacgaccccaccgcccacgccgagatcatggccctgcagcagggcggccagatcgtgcagaactaccggctgctgaacgccaccctgtacgtgaccttcgagccctgcgtgatgtgcgccggcgccatggtgcacagcaggatcaagagactggtctacggcgtgagcaactcaaaaagaggcgccgccggcagcctgctgaacgtgctgaactaccccggcatgaaccaccagatcgagatcaccgccggcgtgatggccaacgagtgcagcgagatgctgtgccagttctatggtatgcgcagagaagtgttcaatgctgagcgtgaggctaggcggctgaaccaacctgatagagctgac

SEQ ID NO: 31 - DNA, 647 bp, synthetic construct
  source 1..647: mol_type = other DNA
ccaaagaagaagcggaaagtcatgagtgagctgaatgatgcttactggatgaaacaggcactcgctttagctcagaaggcccgggaacagggagaagttccagtgggcgctattctggtgctggatgatgaagtgataggacagggatggaatagagccatcaccctgcacgaccccaccgcccacgccgagatcatggccctgcagcagggcggccagatcgtgcagaactaccggctgctgaacgccaccctgtacgtgaccttcgagccctgcgtgatgtgcgccggcgccatggtgcacagcaggatcaagagactggtctacggcgtgagcaactcaaaaagaggcgccgccggcagcctgctgaacgtgctgaactaccccggcatgaaccaccagatcgagatcaccgccggcgtgatggccaacgagtgcagcgagatgctgtgccagttctatggtatgcgcagagaagtgttcaatgctgagcgtgaggctaggcggctgaaccaacctgatagagctgactccggaggatctagcggaggctcctctggctctgagacacctggcacaagcgagagcgcaacacctgaaagcagcgggggcagcagcggggggtcaatcaagaaccaaatcatcgg

SEQ ID NO: 32 - DNA, 20 bp, synthetic construct
  source 1..20: mol_type = other DNA
atcaagaaccaaatcatcgg

SEQ ID NO: 33 - DNA, 21 bp, synthetic construct
  source 1..21: mol_type = other DNA
gactttccgcttcttctttgg

SEQ ID NO: 34 - DNA, 3984 bp, synthetic construct
  source 1..3984: mol_type = other DNA
atgaaacggacagccgacggaagcgagttcgagtcaccaaagaagaagcggaaagtcatgagtgagctgaatgatgcttactggatgaaacaggcactcgctttagctcagaaggcccgggaacagggagaagttccagtgggcgctattctggtgctggatgatgaagtgataggacagggatggaatagagccatcaccctgcacgaccccaccgcccacgccgagatcatggccctgcagcagggcggccagatcgtgcagaactaccggctgctgaacgccaccctgtacgtgaccttcgagccctgcgtgatgtgcgccggcgccatggtgcacagcaggatcaagagactggtctacggcgtgagcaactcaaaaagaggcgccgccggcagcctgctgaacgtgctgaactaccccggcatgaaccaccagatcgagatcaccgccggcgtgatggccaacgagtgcagcgagatgctgtgccagttctatggtatgcgcagagaagtgttcaatgctgagcgtgaggctaggcggctgaaccaacctgatagagctgactccggaggatctagcggaggctcctctggctctgagacacctggcacaagcgagagcgcaacacctgaaagcagcgggggcagcagcggggggtcaatcaagaaccaaatcatcggatatgaagtgaagcttgacctcaacgacaggaagagggcttttgttagggataccttgcggtacttcgcccagacatcggatgtgttccgaaagggcctgatgtgcctgttcgctggcgtcgaccccgagatgataagcggctacctgcccgagggggaatccggcgacctgtggtgcgccgtcaactggttccgcctcgtggatctgtcggagggtcttgtctccgaggagcaggtggtagacgggtcggagctgtgccgcaggttccaagactacgcaggtcatgcgcccgaccggcaggcggagatatacctgactaggaggagcgagggcgatgtccagtacgtttgggccgactgccgtgctggctaccgcagcttctgccgtgaggtgggactgagcccagaccagatggcatttgacgtgcttgcgcttgtggcaaggggctacatcaagttcgacaagggcgaaaacgatgcctgggggtttgtatccgccgtcttcggcgacggcgtcaaggaggacaccaagaacaagattcgcatgctcgagggcatgaggagagcagcacacgccaagccggccacctacgaggagcttcaggaatcggcgctgagggagacgggatgcagcgacatcaagcaaatgatcatggagtacaagtccggtcagcaggacgacaaggaaggcgtcagaaaaagcagcgccggcagtcacgcattcttcgtgaaatacttcttgaggggagccgatcgggtatgcggccccatcggcgagaaggagctggaattgtttgtcagtagctgcgacaagaccctgaagcaaaaaacatcgtgcgacgaggcgccgatcacgcacagtgccgtgtggaagaggtggttcaagaggaggataccgcacaccgtcggttcaatccaggaaccatacagcgttgcgtgcgaccaagccatggccgacataagctctaagaactgcctgaacgcccgcatggtgagctgcccagacagcggctcggtggccgagcgcaggaagaagggcaccaaggcgaagaaggtcgggtcatccggcgtgctcgagatgcaggacaaggtttcgtccctgtcgagcaagggcgttgatcttgcgaagtccgtattcgacagcttcaacgatgctctggacagagaccgcaaggaggacgaggattcctgccggttcgaggtcctcaggcatcacctcggcaagctttccgacctttacgagatttgggtgaagaacgactgcgactccggcataggtctctatctggaggaatacgaaggttcgattaaaaaacagccgaaagaggaactgctgcgtgcgatctacccgcatcgagagtcaataaaggccaaggagttcatggacgcagcgcaccgcaacgacctcatccaaaagatcgagtcccgcaaggcgcacccgactgtgcgtggcaacaggggcgtcggttacggcaactccaagttgaggggcaagataatgccgcagtccaacatgcacaaaggtcgcaaagccggcctgaaccccgagatgtggctcgaggcggatctcctgaacggggagaggtgggagaagcatcacctgaagttccactcgtcgcagttcttcgatcaggtctactgccacaaggacggactgccctacacgaaaatccctggcctgccgaggttggcacggcacggcatgcccatcgggctgtcgataagccccgatgacgttcctctggtgaaccgtgtgtccggcaacggcaggcgttgcccgagggcgaacaagagaaaccttagggccgtcgccaacatcactcacaacgtggaactccacccggagacagccttcgagatacgcagcaacggcgaatacgcaagcatcagccacagggtgcaagatgtcgccaagaagagcatcgaggccggcgatcgaagtcttggctacgaccgaaatcagaccgcacaggacacctacgcagtactgtgtgtcgtcaacgagggaggttatgcccacaggggcaacttggtcgagctcgtcgccgtcggcaagatctcgagcaagagcatgaagcgcaggacggacggctcgatgtacgagtgcgacgacctggcctatgacggcttgccttatgcggagttctccgagtggagggaggaacggaaagcattcatgcatcgcctgatcccgctgctgcctccggcaaccaagaagcttggcagcagcagggagccgatggatctgccgaaggaactcgaggccctgacgcactgcaagtcgctttacgtgtggaaccgcaggttcctgaccatcttccggatcgcactgaagagggccacgaaggaacaggcgcccgatctgttccgccaggagatactcgacatctgtcacgccaatcttagcccgctgagacgaagcagcctgagcaaggacggagttgaatcacttcagaagctgaaaggactcgtcaacgcctacctcagcaaaatgaaggcgaagaagaaagatccactgcttgaggccgacccagagttcgccgagctgttcaaggtaatcaacgatcgtctcaaggcgaaaaggctcgagaaggccaaacgcacagccagcgatatcgtccggctggccaacctgcacggctgctccttcgtctccggcgagtccgacctgccgacgaccagcaaggtcaacaagaaattccagaacgcaagcaacatggactggatggctcgcaaggtcgaggacctcgtcaagagcatgtgcattaggtctggcatcgcctttagaggcatcgacccgtcctacacgagcctgcgtgatccgttacagttcgagaccgacggcaggagcgtcatccgatgccgtttctggaaggcggaaaatggctcggctccggaatatgtcatcgatggtctggtgcgttacacgaagcacgccgtcaagaacatggagcagtcaaggcccctgtcgtccttccacagaggcgggctggccttctgccgcaagtacggcatcgacccagcgagactgacgcccaaggtcgtccgtggcgtgctggcgaggcacgaggtggtatacttgccacgtgccggcggcaggtacttcctcgccacgctgccgctggtggcgggggctcccgtcttcgagtgggatggccagcagatgtatgtcctcgacgccgcagaggtcgctgcgatcaacatcgcactcgaagccataccttccaagctaccgtctggcggctcaaaaagaaccgccgacggcagcgaattcgagcccaagaagaagaggaaagtctaa

SEQ ID NO: 35 - protein, 18 aa, synthetic construct
KRTADGSEFESPKKKRKV

SEQ ID NO: 36 - protein, 20 aa, synthetic construct
AVKRPAATKKAGQAKKKKLD

SEQ ID NO: 37 - protein, 16 aa, synthetic construct
KRPAATKKAGQAKKKK

SEQ ID NO: 38 - protein, 17 aa, synthetic construct
KKTELQTTNAENKTKKL

SEQ ID NO: 39 - protein, 19 aa, synthetic construct
KRGINDRNFWRGENGRKTR

SEQ ID NO: 40 - protein, 16 aa, synthetic construct
RKSGKIAAIVVKRPRK

SEQ ID NO: 41 - protein, 7 aa, synthetic construct
PKKKRKV

SEQ ID NO: 42 - protein, 30 aa, synthetic construct
MDSLLMNRRKFLYQFKNVRWAKGRRETYLC

SEQ ID NO: 43 - protein, 1327 aa, synthetic construct
MKRTADGSEFESPKKKRKVMSELNDAYWMKQALALAQKAREQGEVPVGAILVLDDEVIGQGWNRAITLHDPTAHAEIMALQQGGQIVQNYRLLNATLYVTFEPCVMCAGAMVHSRIKRLVYGVSNSKRGAAGSLLNVLNYPGMNHQIEITAGVMANECSEMLCQFYGMRREVFNAEREARRLNQPDRADSGGSSGGSSGSETPGTSESATPESSGGSSGGSIKNQIIGYEVKLDLNDRKRAFVRDTLRYFAQTSDVFRKGLMCLFAGVDPEMISGYLPEGESGDLWCAVNWFRLVDLSEGLVSEEQVVDGSELCRRFQDYAGHAPDRQAEIYLTRRSEGDVQYVWADCRAGYRSFCREVGLSPDQMAFDVLALVARGYIKFDKGENDAWGFVSAVFGDGVKEDTKNKIRMLEGMRRAAHAKPATYEELQESALRETGCSDIKQMIMEYKSGQQDDKEGVRKSSAGSHAFFVKYFLRGADRVCGPIGEKELELFVSSCDKTLKQKTSCDEAPITHSAVWKRWFKRRIPHTVGSIQEPYSVACDQAMADISSKNCLNARMVSCPDSGSVAERRKKGTKAKKVGSSGVLEMQDKVSSLSSKGVDLAKSVFDSFNDALDRDRKEDEDSCRFEVLRHHLGKLSDLYEIWVKNDCDSGIGLYLEEYEGSIKKQPKEELLRAIYPHRESIKAKEFMDAAHRNDLIQKIESRKAHPTVRGNRGVGYGNSKLRGKIMPQSNMHKGRKAGLNPEMWLEADLLNGERWEKHHLKFHSSQFFDQVYCHKDGLPYTKIPGLPRLARHGMPIGLSISPDDVPLVNRVSGNGRRCPRANKRNLRAVANITHNVELHPETAFEIRSNGEYASISHRVQDVAKKSIEAGDRSLGYDRNQTAQDTYAVLCVVNEGGYAHRGNLVELVAVGKISSKSMKRRTDGSMYECDDLAYDGLPYAEFSEWREERKAFMHRLIPLLPPATKKLGSSREPMDLPKELEALTHCKSLYVWNRRFLTIFRIALKRATKEQAPDLFRQEILDICHANLSPLRRSSLSKDGVESLQKLKGLVNAYLSKMKAKKKDPLLEADPEFAELFKVINDRLKAKRLEKAKRTASDIVRLANLHGCSFVSGESDLPTTSKVNKKFQNASNMDWMARKVEDLVKSMCIRSGIAFRGIDPSYTSLRDPLQFETDGRSVIRCRFWKAENGSAPEYVIDGLVRYTKHAVKNMEQSRPLSSFHRGGLAFCRKYGIDPARLTPKVVRGVLARHEVVYLPRAGGRYFLATLPLVAGAPVFEWDGQQMYVLDAAEVAAINIALEAIPSKLPSGGSKRTADGSEFEPKKKRKV

SEQ ID NO: 44 - protein, 1086 aa, synthetic construct
MIKNQIIGYEVKLDLNDRKRAFVRDTLRYFAQTSDVFRKGLMCLFAGVDPEMISGYLPEGESGDLWCAVNWFRLVDLSEGLVSEERVVDGSELCRRFQDYAGHAPDRQAEIYLTRRSEGDVQYVWADCRAGYRSFCREVGLSPDQMGFDVLALVARGYIKFDKGENDAWGFVSAVFGDGVKEDTKNKIRMLEGMRRAAHAKPATYEELQESALRETGCSDIKQMIREYKSGQQDDKEGVRKSSGGSHAFFVKYFLRGADRVCGPIGEKELELFVSSCDKTLKQKTSCDEAPITHSAVWKRWFKRRIPHTVGSIQEPYSVACDQAMADISSKNCLNARMVSCPDSGSVAERRKKGTKAKKVGSSGVLEMQDKVSSLSSKGVDLAKSVFDSFNDALDRDRKEDEDSCRFEVLRHHLGKLSDLYEIWVKNDCDSGIGLYLEEYEGSIKKQPKEELLRAIYPHRESIKAKEFMDAAHRNDLIQKIESRKAHPTVRGNRGVGYGKSKMRGKIMPQSNMHNGRKAGLNPEMWLEADLLNGERWEKHHLKFHSSQFFDQVYCHKDGLPYTKIPGLPRLARHGMPIGLSISPDDVPLVNRVSGNGRRCPRANKRNLRAVANITHNVELHPETAFEIRSNGEYASISHRVQDVAKKSIEAGDRSLGYARNQTAQDTYAVLCVVNEGGYAHRGNLVELVAVGKISSKSMKRRTDGSMYECDDLAYDGLPYAEFSEWREERKAFMHRLIPLLPPATKKLGSSREPMDLPKELEALTHCKSLYVWNRRFLIIFRVALKRALKEQASNLFRQEILDICHANLSPLRRSSLSKSGVESLQKLKSLVNAYLSKMKAKREDPLLEADPEFAELFKVITERLKAKRLEKAKRTASDIVRLANLHGCSFVSGESDLPTTSKVNKKFQNASNTDWMARKVEDLVKSMCIRSGIAFRGIDPSYTSLRDPLQFETDGRSVIRCRFWKAENGSAPEYVIDGLVRYTKHAVKNMEQSRPLSSFHRGGLAFCRKYGIDPARLTPKVVRGVLARHEVVYLPRAGGRYFLATLPLVAGAPVFEWDGQQMYVLDADEVAAINIALEAIPSKLP

SEQ ID NO: 45 - protein, 1086 aa, synthetic construct
MIKNQIIGYEVKLDLNDRKRAFVRDTLRYFAQTSDVFRKGLMCLFAGVDPEMISGYLPEGESGDLWCAVNWFRLVDLSEGLVSEERVVDGSELCRRFQDYAGHAPDRQAEIYLTRRSEGDVQYVWADCRAGYRSFCREVGLSPDQMGFDVLALVARGYIKFDKGENDAWGFVSAVFGDGVKEDTKNKIRMLEGMRRAAHAKPATYEELQESALRETGCSDIKQMIREYKSGQQDDKEGVRKSSGGSHAFFVKYFLRGADRVCGPIGEKELELFVSSCDKTLKQKTSCDEAPITHSAVWKRWFKRRIPHTVGSIQEPYSVACDQAMADISSKNCLNARMVSCPDSGSVAERRKKGTKAKKVGSSGVLEMQDKVSSLSSKGVDLAKSVFDSFNDALDRDRKEDEDSCRFEVLRHHLGKLSDLYEIWVKNDCDSGIGLYLEEYEGSIKKQPKEELLRAIYPHRESIKAKEFMDAAHRNDLIQKIESRKAHPTVRGNRGVGYGKSKMRGKIMPQSNMHNGRKAGLNPEMWLEADLLNGERWEKHHLKFHSSQFFDQVYCHKDGLPYTKIPGLPRLARHGMPIGLSISPDDVPLVNRVSGNGRRCPRANKRNLRAVANITHNVELHPETAFEIRSNGEYASISHRVQDVAKKSIEAGDRSLGYDRNQTAQDTYAVLCVVNEGGYAHRGNLVELVAVGKISSKSMKRRTDGSMYECADLAYDGLPYAEFSEWREERKAFMHRLIPLLPPATKKLGSSREPMDLPKELEALTHCKSLYVWNRRFLIIFRVALKRALKEQASNLFRQEILDICHANLSPLRRSSLSKSGVESLQKLKSLVNAYLSKMKAKREDPLLEADPEFAELFKVITERLKAKRLEKAKRTASDIVRLANLHGCSFVSGESDLPTTSKVNKKFQNASNTDWMARKVEDLVKSMCIRSGIAFRGIDPSYTSLRDPLQFETDGRSVIRCRFWKAENGSAPEYVIDGLVRYTKHAVKNMEQSRPLSSFHRGGLAFCRKYGIDPARLTPKVVRGVLARHEVVYLPRAGGRYFLATLPLVAGAPVFEWDGQQMYVLDADEVAAINIALEAIPSKLP

SEQ ID NO: 46 - protein, 1086 aa, synthetic construct
MIKNQIIGYEVKLDLNDRKRAFVRDTLRYFAQTSDVFRKGLMCLFAGVDPEMISGYLPEGESGDLWCAVNWFRLVDLSEGLVSEERVVDGSELCRRFQDYAGHAPDRQAEIYLTRRSEGDVQYVWADCRAGYRSFCREVGLSPDQMGFDVLALVARGYIKFDKGENDAWGFVSAVFGDGVKEDTKNKIRMLEGMRRAAHAKPATYEELQESALRETGCSDIKQMIREYKSGQQDDKEGVRKSSGGSHAFFVKYFLRGADRVCGPIGEKELELFVSSCDKTLKQKTSCDEAPITHSAVWKRWFKRRIPHTVGSIQEPYSVACDQAMADISSKNCLNARMVSCPDSGSVAERRKKGTKAKKVGSSGVLEMQDKVSSLSSKGVDLAKSVFDSFNDALDRDRKEDEDSCRFEVLRHHLGKLSDLYEIWVKNDCDSGIGLYLEEYEGSIKKQPKEELLRAIYPHRESIKAKEFMDAAHRNDLIQKIESRKAHPTVRGNRGVGYGKSKMRGKIMPQSNMHNGRKAGLNPEMWLEADLLNGERWEKHHLKFHSSQFFDQVYCHKDGLPYTKIPGLPRLARHGMPIGLSISPDDVPLVNRVSGNGRRCPRANKRNLRAVANITHNVELHPETAFEIRSNGEYASISHRVQDVAKKSIEAGDRSLGYDRNQTAQDTYAVLCVVNEGGYAHRGNLVELVAVGKISSKSMKRRTDGSMYECDDLAYDGLPYAEFSEWREERKAFMHRLIPLLPPATKKLGSSREPMDLPKELEALTHCKSLYVWNRRFLIIFRVALKRALKEQASNLFRQEILDICHANLSPLRRSSLSKSGVESLQKLKSLVNAYLSKMKAKREDPLLEADPEFAELFKVITERLKAKRLEKAKRTASDIVRLANLHGCSFVSGASDLPTTSKVNKKFQNASNTDWMARKVEDLVKSMCIRSGIAFRGIDPSYTSLRDPLQFETDGRSVIRCRFWKAENGSAPEYVIDGLVRYTKHAVKNMEQSRPLSSFHRGGLAFCRKYGIDPARLTPKVVRGVLARHEVVYLPRAGGRYFLATLPLVAGAPVFEWDGQQMYVLDADEVAAINIALEAIPSKLP

SEQ ID NO: 47 - protein, 1086 aa, synthetic construct
MIKNQIIGYEVKLDLNDRKRAFVRDTLRYFAQTSDVFRKGLMCLFAGVDPEMISGYLPEGESGDLWCAVNWFRLVDLSEGLVSEERVVDGSELCRRFQDYAGHAPDRQAEIYLTRRSEGDVQYVWADCRAGYRSFCREVGLSPDQMGFDVLALVARGYIKFDKGENDAWGFVSAVFGDGVKEDTKNKIRMLEGMRRAAHAKPATYEELQESALRETGCSDIKQMIREYKSGQQDDKEGVRKSSGGSHAFFVKYFLRGADRVCGPIGEKELELFVSSCDKTLKQKTSCDEAPITHSAVWKRWFKRRIPHTVGSIQEPYSVACDQAMADISSKNCLNARMVSCPDSGSVAERRKKGTKAKKVGSSGVLEMQDKVSSLSSKGVDLAKSVFDSFNDALDRDRKEDEDSCRFEVLRHHLGKLSDLYEIWVKNDCDSGIGLYLEEYEGSIKKQPKEELLRAIYPHRESIKAKEFMDAAHRNDLIQKIESRKAHPTVRGNRGVGYGKSKMRGKIMPQSNMHNGRKAGLNPEMWLEADLLNGERWEKHHLKFHSSQFFDQVYCHKDGLPYTKIPGLPRLARHGMPIGLSISPDDVPLVNRVSGNGRRCPRANKRNLRAVANITHNVELHPETAFEIRSNGEYASISHRVQDVAKKSIEAGDRSLGYDRNQTAQDTYAVLCVVNEGGYAHRGNLVELVAVGKISSKSMKRRTDGSMYECDDLAYDGLPYAEFSEWREERKAFMHRLIPLLPPATKKLGSSREPMDLPKELEALTHCKSLYVWNRRFLIIFRVALKRALKEQASNLFRQEILDICHANLSPLRRSSLSKSGVESLQKLKSLVNAYLSKMKAKREDPLLEADPEFAELFKVITERLKAKRLEKAKRTASDIVRLANLHGCSFVSGESDLPTTSKVNKKFQNASNTDWMARKVEDLVKSMCIRSGIAFRGIDPSYTSLRDPLQFETDGRSVIRCRFWKAENGSAPEYVIDGLVRYTKHAVKNMEQSRPLSSFHRGGLAFCRKYGIDPARLTPKVVRGVLARHEVVYLPRAGGRYFLATLPLVAGAPVFEWDGQQMYVLDAAEVAAINIALEAIPSKLP

SEQ ID NO: 48 - DNA, 20 bp, synthetic construct
  source 1..20: mol_type = other DNA
tagaagggatatacaaagtg

SEQ ID NO: 49 - DNA, 45 bp, synthetic construct
  source 1..45: mol_type = other DNA
tatccatcgtgccgcctcttggcactagaagggatatacaaagtg

SEQ ID NO: 50 - DNA, 49 bp, synthetic construct
  source 1..49: mol_type = other DNA
cacctatccatcgtgccgcctcttggcactagaagggatatacaaagtg

SEQ ID NO: 51 - DNA, 49 bp, synthetic construct
  source 1..49: mol_type = other DNA
aaaacactttgtatatcccttctagtgccaagaggcggcacgatggata

SEQ ID NO: 52 - DNA, 7665 bp, synthetic construct
  source 1..7665: mol_type = other DNA
taacgcaggaaagaacatgtgagcaaaaggccagcaaaaggccaggaaccgtaaaaaggccgcgttgctggcgtttttccataggctccgcccccctgacgagcatcacaaaaatcgacgctcaagtcagaggtggcgaaacccgacaggactataaagataccaggcgtttccccctggaagctccctcgtgcgctctcctgttccgaccctgccgcttaccggatacctgtccgcctttctcccttcgggaagcgtggcgctttctcatagctcacgctgtaggtatctcagttcggtgtaggtcgttcgctccaagctgggctgtgtgcacgaaccccccgttcagcccgaccgctgcgccttatccggtaactatcgtcttgagtccaacccggtaagacacgacttatcgccactggcagcagccactggtaacaggattagcagagcgaggtatgtaggcggtgctacagagttcttgaagtggtggcctaactacggctacactagaaggacagtatttggtatctgcgctctgctgaagccagttaccttcggaaaaagagttggtagctcttgatccggcaaacaaaccaccgctggtagcggtggtttttttgtttgcaagcagcagattacgcgcagaaaaaaaggatctcaagaagatcctttgatcttttctacggggtctgacgctcagtggaacgaaaactcacgttaagggattttggtcatgagattatcaaaaaggatcttcacctagatccttttaaattaaaaatgaagttttaaatcaatctaaagtatatatgagtaacctgaggctatggcagggcctgccgccccgacgttggctgcgagccctgggccttcacccgaacttggggggtggggtggggaaaaggaagaaacgcgggcgtattggccccaatggggtctcggtggggtatcgacagagtgccagccctgggaccgaaccccgcgtttatgaacaaacgacccaacaccgtgcgttttattctgtctttttattgccgtcatagcgcgggttccttccggtattgtctccttccgtgtttcagttagcctccccctagggtgggcgaagaactccagcatgagatccccgcgctggaggatcatccagccggcgtcccggaaaacgattccgaagcccaacctttcatagaaggcggcggtggaatcgaaatctcgtgatggcaggttgggcgtcgcttggtcggtcatttcgaaccccagagtcccgctcagaagaactcgtcaagaaggcgatagaaggcgatgcgctgcgaatcgggagcggcgataccgtaaagcacgaggaagcggtcagcccattcgccgccaagctcttcagcaatatcacgggtagccaacgctatgtcctgatagcggtccgccacacccagccggccacagtcgatgaatccagaaaagcggccattttccaccatgatattcggcaagcaggcatcgccatgggtcacgacgagatcctcgccgtcgggcatgctcgccttgagcctggcgaacagttcggctggcgcgagcccctgatgctcttcgtccagatcatcctgatcgacaagaccggcttccatccgagtacgtgctcgctcgatgcgatgtttcgcttggtggtcgaatgggcaggtagccggatcaagcgtatgcagccgccgcattgcatcagccatgatggatactttctcggcaggagcaaggtgagatgacaggagatcctgccccggcacttcgcccaatagcagccagtcccttcccgcttcagtgacaacgtcgagcacagctgcgcaaggaacgcccgtcgtggccagccacgatagccgcgctgcctcgtcttgcagttcattcagggcaccggacaggtcggtcttgacaaaaagaaccgggcgcccctgcgctgacagccggaacacggcggcatcagagcagccgattgtctgttgtgcccagtcatagccgaatagcctctccacccaagcggccggagaacctgcgtgcaatccatcttgttcaatcatgcgaaacgatcctcatcctgtctcttgatcgatctttgcaaaagcctaggcctccaaaaaagcctcctcactacttctggaatagctcagaggccgaggcggcctcggcctctgcataaataaaaaaaattagtcagccatggggcggagaatgggcggaactgggcggagttaggggcgggatgggcggagttaggggcgggactatggttgctgactaattgagatgcatgctttgcatacttctgcctgctggggagcctggggactttccacacctggttgctgactaattgagatgcatgctttgcatacttctgcctgctggggagcctggggactttccacaccctaactgacacacattccacagctggttctttccgcctcaggactcttcctttttcaatattattgaagcatttatcagggttattgtctcatgagcggatacatatttgaatgtatttagaaaaataaacaaataggggttccgcgcacatttccccgaaaagtgccacctgacgcgccctgtagcggcgcattaagcgcggcgggtgtggtggttacgcgcagcgtgaccgctacacttgccagcgccctagcgcccgctcctttcgctttcttcccttcctttctcgccacgttcgccggctttccccgtcaagctctaaatcgggggctccctttagggttccgatttagtgctttacggcacctcgaccccaaaaaacttgattagggtgatggttcacgtagtgggccatcgccctgatagacggtttttcgccctttgacgttggagtccacgttctttaatagtggactcttgttccaaactggaacaacactcaaccctatctcggtctattcttttgatttataagggattttgccgatttcggcctattggttaaaaaatgagctgatttaacaaaaatttaacgcgaattttaacaaaatattaacgcttacaatttacgcgttaagatacattgatgagtttggacaaaccacaactagaatgcagtgaaaaaaatgctttatttgtgaaatttgtgatgctattgctttatttgtaaccattataagctgcaataaacaagttaacaacaacaattgcattcattttatgtttcaggttcagggggaggtgtgggaggttttttaaagcaagtaaaacctctacaaatgtggtatggctgattatgatcagttatctagatccggtggatcccgggttacaatttggactttccgcccttcttggcctttatgaggatctctctgatttttcttgcgtcgagttttccggtaagacctttcggtacttcgtccacaaacacaactcctccgcgcaactttttcgcggttgttacttgactggcgacgtaatccacgatctctttttccgtcatcgtctttccgtgctccaaaacaacaacggcggcgggaagttcaccggcgtcatcgtcgggaagacctgccacgcccgcgtcgaagatgttggggtgttgtaacaatatcgattccaattcagcgggggccacctgatatcctttgtatttaattaaagacttcaagcggtcaactatgaagaagtgttcgtcttcgtcccagtaagctatgtctccagaatgtagccatccatccttgtcaatcaaggcgttggtcgcttccggattgtttacataaccggacataatcataggtcctctgacacataattcgcctctctgattaacgcccagcgttttcccggtatccagatccacaaccttcgcttcaaaaaatggaacaactttaccgaccgcgcccggtttatcatccccctcgggtgtaatcagaatagctgatgtagtctcagtgagcccatatccttgtcgtatccctggaagatggaagcgttttgcaaccgcttccccgacttctttcgaaagaggtgcgcccccagaagcaatttcgtgtaaattagataaatcgtatttgtcaatcagagtgcttttggcgaagaatgaaaatagggttggtactagcaacgcactttgaattttgtaatcctgaagggatcgtaaaaacagctcttcttcaaatctatacattaagacgactcgaaatccacatatcaaatatccgagtgtagtaaacattccaaaaccgtgatggaatggaacaacacttaaaatcgcagtatccggaatgatttgattgccaaaaataggatctctggcatgcgagaatctgacgcaggcagttctatgcggaagggccacacccttaggtaacccagtagatccagaggaattcattatcagtgcaattgttttgtcacgatcaaaggactctggtacaaaatcgtattcattaaaaccgggaggtagatgagatgtgacgaacgtgtacatcgactgaaatccctggtaatccgttttagaatccatgataataattttctggattattggtaattttttttgcacgttcaaaattttttgcaacccctttttggaaacaaacactacggtaggctgcgaaatgttcatactgttgagcaattcacgttcattataaatgtcgttcgcgggcgcaactgcaactccgataaataacgcgcccaacaccggcataaagaattgaagagagttttcactgcatacgacgattctgtgatttgtattcagcccatatcgtttcatagcttctgccaaccgaacggacatttcgaagtattccgcgtacgtgatgttcacctcgatatgtgcatctgtaaaagcaattgttccaggaaccagggcgtatctcttcatagccttatgcagttgctctccagcggttccatcctctagaggatagaatggcgccgggcctttctttatgtttttggcgtcttccatgctagcggatctgacggttcactaaaccagctctgcttatatagacctcccaccgtacacgcctaccgcccatttgcgtcaatggggcggagttgttacgacattttggaaagtcccgttgattttggtgccaaaacaaactcccattgacgtcaatggggtggagacttggaaatccccgtgagtcaaaccgctatccacgcccattgatgtactgccaaaaccgcatcaccatggtaatagcgatgactaatacgtagatgtactgccaagtaggaaagtcccataaggtcatgtactgggcataatgccaggcgggccatttaccgtcattgacgtcaatagggggcgtacttggcatatgatacacttgatgtactgccaagtgggcagtttaccgtaaatactccacccattgacgtcaatggaaagtccctattggcgttactatgggaacatacgtcattattgacgtcaatgggcgggggtcgttgggcggtcagccaggcgggccatttaccgtaagttatgtaacgcggaactccatatatgggctatgaactaatgaccccgtaattgattactattaggcacgtgggctccggtgcccgtcagtgggcagagcgcacatcgcccacagtccccgagaagttggggggaggggtcggcaattgaaccggtgcctagagaaggtggcgcggggtaaactgggaaagtgatgtcgtgtactggctccgcctttttcccgagggtgggggagaaccgtatataagtgcagtagtcgccgtgaacgttctttttcgcaacgggtttgccgccagaacacaggtaagtgccgtgtgtggttcccgcgggcctggcctctttacgggttatggcccttgcgtgccttgaattacttccacctggctgcagtacgtgattcttgatcccgagcttcgggttggaagtgggtgggagagttcgaggccttgcgcttaaggagccccttcgcctcgtgcttgagttgaggcctggcctgggcgctggggccgccgcgtgcgaatctggtggcaccttcgcgcctgtctcgctgctttcgataagtctctagccatttaaaatttttgatgacctgctgcgacgctttttttctggcaagatagtcttgtaaatgcgggccaagatctgcacactggtatttcggtttttggggccgcgggcggcgacggggcccgtgcgtcccagcgcacatgttcggcgaggcggggcctgcgagcgcggccaccgagaatcggacgggggtagtctcaagctggccggcctgctctggtgcctggcctcgcgccgccgtgtatcgccccgccctgggcggcaaggctggcccggtcggcaccagttgcgtgagcggaaagatggccgcttcccggccctgctgcagggagctcaaaatggaggacgcggcgctcgggagagcgggcgggtgagtcacccacacaaaggaaaagggcctttccgtcctcagccgtcgcttcatgtgactccactgagtaccgggcgccgtccaggcacctcgattagttctcgagcttttggagtacgtcgtctttaggttggggggaggggttttatgcgatggagtttccccacactgagtgggtggagactgaagttaggccagcttggcacttgatgtaattctccttggaatttgccctttttgagtttggatcttggttcattctcaagcctcagacagtggttcaaagtttttttcttccatttcaggtgtcgtgatctagagactagtcccctagccatgggatcccagtccggcgtcttcacactcgaagatttcgttggggactggcgacagacagccggctacaacctggaccaagtccttgaacagggaggtgtgtccagtttgtttcagaatcttttgtagaagggatatacaaagtgcgggtgacggctacaacctggaccaagtccttgaacagggaggtgtgtccagtttgtttcagaatctcggggtgtccgtaactccgatccaaaggattgtcctgagcggtgaaaatgggctgaagatcgacatccatgtcatcatcccgtatgaaggtctgagcggcgaccaaatgggccagatcgaaaaaatttttaaggtggtgtaccctgtggatgatcatcactttaaggtgatcctgcactatggcacactggtaatcgacggggttacgccgaacatgatcgactatttcggacggccgtatgaaggcatcgccgtgttcgacggcaaaaagatcactgtaacagggaccctgtggaacggcaacaaaattatcgacgagcgcctgatcaaccccgacggctccctgctgttccgagtaaccatcaacggagtgaccggctggcggctgtgcgaacgcattctggcgtaagtcgactgtgccttctagttgccagccatctgttgtttgcccctcccccgtgccttccttgaccctggaaggtgccactcccactgtcctttcctaataaaatgaggaaattgcatcgcattgtctgagtaggtgtcattctattctggggggtggggtggggcaggacagcaagggggaggattgggaagacaatagcaggcatgctggggatgcggtgggctctatggctcaagcttataactaatgcatggcggtaatacggttatccacagaatcagggga

SEQ ID NO: 53 - DNA, 36 bp, synthetic construct
  source 1..36: mol_type = other DNA
tttgtagaagggatatacaaagtggaaatcgggtga

SEQ ID NO: 54 - protein, 180 aa, synthetic construct
MYNAPRFFCRSAAVSDHEFNDEYWMRHALTLAKRAREEGEVPVGAVLVLNNQVIGEGWNRAIGLHDPTAHAEIMALRQGGLVLQNYRLIDATLYVTFEPCVMCAGAMVHSRISRLVFGVRNSKRGAAGSLINVLNYPGMNHRVEITEGILAESCSAMLCDFYRWPREVFNALKKARQEEG

SEQ ID NO: 55 - protein, 167 aa, synthetic construct
MSEVEFSHEYWMRHALTLAKRARDEREVPVGAVLVLNNRVIGEGWNRAIGLHDPTAHAEIMALRQGGLVMQNYRLIDATLYVTFEPCVMCAGAMIHSRIGRVVFGVRNSKRGAAGSLMNVLNYPGMNHRVEITEGILADECAALLCDFYRMPRQVFNAQKKAQSSIN

SEQ ID NO: 56 - DNA, 38 bp, synthetic construct
  source 1..38: mol_type = other DNA
cacttcgtaaggtcgcttgacaagaccctgaagcaaaa

SEQ ID NO: 57 - DNA, 38 bp, synthetic construct
  source 1..38: mol_type = other DNA
aagcgaccttacgaagtgttccagctccttctcgccga

SEQ ID NO: 58 - DNA, 15 bp, synthetic construct
  source 1..15: mol_type = other DNA
tagaagggatataca

SEQ ID NO: 59 - DNA, 18 bp, synthetic construct
  source 1..18: mol_type = other DNA
tagaagggatatacaaag

SEQ ID NO: 60 - DNA, 19 bp, synthetic construct
  source 1..19: mol_type = other DNA
tagaagggatatacaaagt

SEQ ID NO: 61 - DNA, 21 bp, synthetic construct
  source 1..21: mol_type = other DNA
tagaagggatatacaaagtgg

SEQ ID NO: 62 - DNA, 22 bp, synthetic construct
  source 1..22: mol_type = other DNA
tagaagggatatacaaagtgga

SEQ ID NO: 63 - DNA, 23 bp, synthetic construct
  source 1..23: mol_type = other DNA
tagaagggatatacaaagtggaa

SEQ ID NO: 64 - DNA, 25 bp, synthetic construct
  source 1..25: mol_type = other DNA
tagaagggatatacaaagtggaaat